European Patent Specification EP 3 562 504 B1, published April 19, 2023. Title: Plant protein signal sequence as adjuvant in DNA vaccines. Applicant: ENEA ISTITUTI FISIOTERAPICI OSPITALIERI. The sequence listing filed with the application follows.

SEQUENCE LISTING (36 sequences)

SEQ ID NO: 1 - protein, 29 aa, Phaseolus vulgaris
MTQFNIPVTMSSSLSIILVILVSLRTALS

SEQ ID NO: 2 - DNA, 35 bp, Artificial Sequence
  primer
ggccggtaccatcatgactcaattcaatatccaag

SEQ ID NO: 3 - DNA, 39 bp, Artificial Sequence
  primer
tgtaggtgtatctccatgcattgagagtgcagttctcaa

SEQ ID NO: 4 - DNA, 39 bp, Artificial Sequence
  primer
ttgagaactgcactctcaatgcatggagatacacctaca

SEQ ID NO: 5 - DNA, 39 bp, Artificial Sequence
  primer
ttctcgacttgcggccgcttatggtttctgagaacagat

SEQ ID NO: 6 - DNA, 35 bp, Artificial Sequence; identical to SEQ ID NO: 2
  primer

SEQ ID NO: 7 - DNA, 39 bp, Artificial Sequence
  primer
ctgtgttgtgctagctggtggtttctgagaacagatggg

SEQ ID NO: 8 - DNA, 39 bp, Artificial Sequence
  primer
atctgttctcagaaaccaccagctagcacaacacagccc

SEQ ID NO: 9 - DNA, 39 bp, Artificial Sequence
  primer
ttctcgacttgcggccgcttatggtggtggtagagtgac

SEQ ID NO: 10 - DNA, 35 bp, Artificial Sequence; identical to SEQ ID NO: 2
  primer

SEQ ID NO: 11 - DNA, 42 bp, Artificial Sequence
  primer
gctagctggaggtccgggtcctggtttctgagaacagatggg

SEQ ID NO: 12 - DNA, 42 bp, Artificial Sequence
  primer
cagaaaccaggacccggacctccagctagcacaacacagccc

SEQ ID NO: 13 - DNA, 39 bp, Artificial Sequence; identical to SEQ ID NO: 9
  primer

SEQ ID NO: 14 - DNA, 32 bp, Artificial Sequence
  primer
ggccggatccatcatgcgtcacaaacgttcag

SEQ ID NO: 15 - DNA, 32 bp, Artificial Sequence
  primer
ggccctgcagttaaaatgtatccatcggaatt

SEQ ID NO: 16 - DNA, 35 bp, Artificial Sequence
  primer
ggccggatccatcatgactcaattcaatatccaag

SEQ ID NO: 17 - DNA, 37 bp, Artificial Sequence
  primer
tgaacgtttgtggacgcattgagagtgcagttctcaa

SEQ ID NO: 18 - DNA, 36 bp, Artificial Sequence
  primer
ttgagaactgcactctcaatgcgtcacaaacgttca

SEQ ID NO: 19 - DNA, 32 bp, Artificial Sequence; identical to SEQ ID NO: 15
  primer

SEQ ID NO: 20 - DNA, 35 bp, Artificial Sequence; identical to SEQ ID NO: 16
  primer

SEQ ID NO: 21 - DNA, 37 bp, Artificial Sequence; identical to SEQ ID NO: 17
  primer

SEQ ID NO: 22 - DNA, 36 bp, Artificial Sequence; identical to SEQ ID NO: 18
  primer

SEQ ID NO: 23 - DNA, 32 bp, Artificial Sequence
  primer
ggccctgcagttatggtttctgagaacagatg

SEQ ID NO: 24 - protein, 9 aa, Human papillomavirus type 16
RAHYNIVTF

SEQ ID NO: 25 - protein, 4 aa, Artificial Sequence
  peptide linker
GPGP

SEQ ID NO: 26 - protein, 98 aa, Artificial Sequence
  HPV16 E7 protein
MHGDTPTLHEYMLDLQPETTDLYCYEQLNDSSEEEDEIDGPAGQAEPDRAHYNIVTFCCKCDSTLRLCVQSTHVDIRTLEDLLMGTLGIVCPICSQKP

SEQ ID NO: 27 - protein, 98 aa, Artificial Sequence
  E7GGG (or E7*) protein from HPV16 E7 mutagenenis
MHGDTPTLHEYMLDLQPETTGLYGYGQLNDSSEEEDEIDGPAGQAEPDRAHYNIVTFCCKCDSTLRLCVQSTHVDIRTLEDLLMGTLGIVCPICSQKP

SEQ ID NO: 28 - protein, 201 aa, Artificial Sequence
  HPV16 L2(1-200) fragment protein optimized for Chlamydomonas rehinardtii codon usage
MRHKRSAKRTKRASATQLYKTCKQAGTCPPDIIPKVEGKTIAEQILQYGSMGVFFGGLGIGTGSGTGGRTGYIPLGTRPPTATDTLAPVRPPLTVDPVGPSDPSIVSLVEETSFIDAGAPTSVPSIPPDVSGFSITTSTDTTPAILDINNTVTTVTTHNNPTFTDPSVLQPPTPAETGGHFTLSSSTISTHNYEEIPMDTF

SEQ ID NO: 29 - protein, 235 aa, Artificial Sequence
  CP protein
MPASTTQPIGSTTSTTTKTAGATPATASGLFTIPDGDFFSTARAIVASNAVATNEDLSKIEAIWKDMKVPTDTMAQAAWDLVRHCADVGSSAQTEMIDTGPYSNGISRARLAAAIKEVCTLRQFCMKYAPVVWNWMLTNNSPPANWQAQGFKPEHKFAAFDFFNGVTNPAAIMPKEGLIRPPSEAEMNAAQTAAFVKITKARAQSNDFASLDAAVTRGRITGTTTAEAVVTLPPP

SEQ ID NO: 30 - protein, 360 aa, Artificial Sequence
  protein obtained by the fusion of SEQ ID NO:1, SEQ ID NO:27 and SEQ ID NO:29
MTQFNIPVTMSSSLSIILVILVSLRTALSHGDTPTLHEYMLDLQPETTGLYGYGQLNDSSEEEDEIDGPAGQAEPDRAHYNIVTFCCKCDSTLRLCVQSTHVDIRTLEDLLMGTLGIVCPICSQKPPASTTQPIGSTTSTTTKTAGATPATASGLFTIPDGDFFSTARAIVASNAVATNEDLSKIEAIWKDMKVPTDTMAQAAWDLVRHCADVGSSAQTEMIDTGPYSNGISRARLAAAIKEVCTLRQFCMKYAPVVWNWMLTNNSPPANWQAQGFKPEHKFAAFDFFNGVTNPAAIMPKEGLIRPPSEAEMNAAQTAAFVKITKARAQSNDFASLDAAVTRGRITGTTTAEAVVTLPPP

SEQ ID NO: 31 - protein, 365 aa, Artificial Sequence
  protein obtained by the fusion of SEQ ID NO:1, SEQ ID NO:27, SEQ ID NO:25 and SEQ ID NO:29
MTQFNIPVTMSSSLSIILVILVSLRTALSMHGDTPTLHEYMLDLQPETTGLYGYGQLNDSSEEEDEIDGPAGQAEPDRAHYNIVTFCCKCDSTLRLCVQSTHVDIRTLEDLLMGTLGIVCPICSQKPGPGPPASTTQPIGSTTSTTTKTAGATPATASGLFTIPDGDFFSTARAIVASNAVATNEDLSKIEAIWKDMKVPTDTMAQAAWDLVRHCADVGSSAQTEMIDTGPYSNGISRARLAAAIKEVCTLRQFCMKYAPVVWNWMLTNNSPPANWQAQGFKPEHKFAAFDFFNGVTNPAAIMPKEGLIRPPSEAEMNAAQTAAFVKITKARAQSNDFASLDAAVTRGRITGTTTAEAVVTLPPP

SEQ ID NO: 32 - protein, 326 aa, Artificial Sequence
  protein obtained by the fusion of SEQ ID NO:1, SEQ ID NO:28 and SEQ ID NO:26
MTQFNIPVTMSSSLSIILVILVSLRTALSRHKRSAKRTKRASATQLYKTCKQAGTCPPDIIPKVEGKTIAEQILQYGSMGVFFGGLGIGTGSGTGGRTGYIPLGTRPPTATDTLAPVRPPLTVDPVGPSDPSIVSLVEETSFIDAGAPTSVPSIPPDVSGFSITTSTDTTPAILDINNTVTTVTTHNNPTFTDPSVLQPPTPAETGGHFTLSSSTISTHNYEEIPMDTFHGDTPTLHEYMLDLQPETTGLYGYGQLNDSSEEEDEIDGPAGQAEPDRAHYNIVTFCCKCDSTLRLCVQSTHVDIRTLEDLLMGTLGIVCPICSQKP

SEQ ID NO: 33 - protein, 332 aa, Artificial Sequence
  protein obtained by the fusion of SEQ ID NO:27 and SEQ ID NO:29
MHGDTPTLHEYMLDLQPETTGLYGYGQLNDSSEEEDEIDGPAGQAEPDRAHYNIVTFCCKCDSTLRLCVQSTHVDIRTLEDLLMGTLGIVCPICSQKPPASTTQPIGSTTSTTTKTAGATPATASGLFTIPDGDFFSTARAIVASNAVATNEDLSKIEAIWKDMKVPTDTMAQAAWDLVRHCADVGSSAQTEMIDTGPYSNGISRARLAAAIKEVCTLRQFCMKYAPVVWNWMLTNNSPPANWQAQGFKPEHKFAAFDFFNGVTNPAAIMPKEGLIRPPSEAEMNAAQTAAFVKITKARAQSNDFASLDAAVTRGRITGTTTAEAVVTLPPP

SEQ ID NO: 34 - protein, 336 aa, Artificial Sequence
  protein obtained by the fusion of SEQ ID NO:27, SEQ ID NO:25 and SEQ ID NO:29
MHGDTPTLHEYMLDLQPETTGLYGYGQLNDSSEEEDEIDGPAGQAEPDRAHYNIVTFCCKCDSTLRLCVQSTHVDIRTLEDLLMGTLGIVCPICSQKPGPGPPASTTQPIGSTTSTTTKTAGATPATASGLFTIPDGDFFSTARAIVASNAVATNEDLSKIEAIWKDMKVPTDTMAQAAWDLVRHCADVGSSAQTEMIDTGPYSNGISRARLAAAIKEVCTLRQFCMKYAPVVWNWMLTNNSPPANWQAQGFKPEHKFAAFDFFNGVTNPAAIMPKEGLIRPPSEAEMNAAQTAAFVKITKARAQSNDFASLDAAVTRGRITGTTTAEAVVTLPPP

SEQ ID NO: 35 - protein, 127 aa, Artificial Sequence
  protein obtained by the fusion of SEQ ID NO:1 and SEQ ID NO:27
MTQFNIPVTMSSSLSIILVILVSLRTALSMHGDTPTLHEYMLDLQPETTGLYGYGQLNDSSEEEDEIDGPAGQAEPDRAHYNIVTFCCKCDSTLRLCVQSTHVDIRTLEDLLMGTLGIVCPICSQKP

SEQ ID NO: 36 - protein, 229 aa, Artificial Sequence
  protein obtained by the fusion of SEQ ID NO:1 and SEQ ID NO:28
MTQFNIPVTMSSSLSIILVILVSLRTALSRHKRSAKRTKRASATQLYKTCKQAGTCPPDIIPKVEGKTIAEQILQYGSMGVFFGGLGIGTGSGTGGRTGYIPLGTRPPTATDTLAPVRPPLTVDPVGPSDPSIVSLVEETSFIDAGAPTSVPSIPPDVSGFSITTSTDTTPAILDINNTVTTVTTHNNPTFTDPSVLQPPTPAETGGHFTLSSSTISTHNYEEIPMDTF